European Patent Specification EP 4 291 647 B1, published June 18, 2025. Title: Subtilisin variants and their use. Applicant: Fresenius Kabi iPSUM Srl. The sequence listing filed with the application follows.

SEQUENCE LISTING (45 sequences)

SEQ ID NO: 1 - DNA, 1149 bp, Bacillus amyloliquefaciens
gtgagaggcaaaaaagtatggatcagtttgctgtttgctttagcgttaatctttacgatggcgttcggcagcacatcctctgcccaggcggcagggaaatcaaacggggaaaagaaatatattgtcgggtttaaacagacaatgagcacgatgagcgccgctaagaagaaagatgtcatttctgaaaaaggcgggaaagtgcaaaagcaattcaaatatgtagacgcagcttcagctacattaaacgaaaaagctgtaaaagaattgaaaaaagacccgagcgtcgcttacgttgaagaagatcacgtagcacatgcgtacgcgcagtccgtgccttacggcgtatcacaaattaaagcccctgctctgcactctcaaggctacactggatcaaatgttaaagtagcggttatcgacagcggtatcgattcttctcatcctgatttaaaggtagcaggcggagccagcatggttccttctgaaacaaatcctttccaagacaacaactctcacggaactcacgttgccggcacagttgcggctcttaataactcaatcggtgtattaggcgttgcgccaagcgcatcactttacgctgtaaaagttctcggtgctgacggttccggccaatacagctggatcattaacggaatcgagtgggcgatcgcaaacaatatggacgttattaacatgagcctcggcggaccttctggttctgctgctttaaaagcggcagttgataaagccgttgcatccggcgtcgtagtcgttgcggcagccggtaacgaaggcacttccggcagctcaagcacagtgggctaccctggtaaatacccttctgtcattgcagtaggcgctgttgacagcagcaaccaaagagcatctttctcaagcgtaggacctgagcttgatgtcatggcacctggcgtatctatccaaagcacgcttcctggaaacaaatacggggcgtacaacggtacgtcaatggcatctccgcacgttgccggagcggctgctttgattctttctaagcacccgaactggacaaacactcaagtccgcagcagtttagaaaacaccactacaaaacttggtgattctttctactatggaaaagggctgatcaacgtacaggcggcagctcagtaa

SEQ ID NO: 2 - protein, 275 aa, Bacillus amyloliquefaciens [sequence omitted]

SEQ ID NO: 3 - protein, 272 aa, Artificial Sequence
  subtilisin BPN' variant of the invention
  VARIANT (87)..(87): L96 position
  VARIANT (90)..(90): D99 position
  VARIANT (214)..(214): A223 position
  VARIANT (215)..(215): S224 position
AQSVPYGVSQIKAPALHSQGYTGSNVKVAVIDSGIDSSHPDLKVAGGASMVPSETNPFQDNNSHGTHVAGTVAAVAPSASLYAVKVXGAXGSGQYSWIINGIEWAIANNMDVINMSLGGPSGSAALKAAVDKAVASGVVVVAAAGNEGTSGSSSTVGYPGKYPSVIAVGAVDSSNQRASFSSVGPELDVMAPGVSIQSTLPGNKYGAYNGTCMXXPHVAGAAALILSKHPNWTNTQVRSSLENTTTKLGDSFYYGKGLINVQAAAQHHHHHH

SEQ ID NO: 4 - protein, 272 aa, Artificial Sequence
  Reference enzyme Ptl-84
AKCVSYGVAQIKAPALHSQGYTGSNVKVAVLDSGIDSSHPDLNVAGGASFVPSETNPFQDNASHGTHVAGTVLAVAPSASLYAVKVLGADGSGQYSWIINGIEWAIANNMDVINMSLGGPSGSAALKAAVDKAVASGVVVVAAAGNNGTSGSSSTVEYPAKYPSVIAVGAVDSSNQRAPWSSVGPELDVMAPGVSICSTLPGGKYGAHDGTCPASNHVAGAAALILSKHPNWTNTQVRSSLENTATKLGDSFYYGKGLINVEAAAQHHHHHH

SEQ ID NO: 5 - protein, 272 aa, Artificial Sequence
  Reference enzyme Ptl-79
AKCVSYGVAQIKAPALHSQGYTGSNVKVAVLDSGIDSSHPDLNVAGGASFVPSETNPFQDNNSHGTHVAGTVLAVAPSASLYAVKVLGADGSGQYSWVINGIEWAIANNMDVINMSLGGPSGSAALKAAVDKAVASGVVVVAAAGNSGTSGSSSTVSYPAKYPSVIAVGAVDSSNQRAPWSSVGPELDVMAPGVSICSTLPGGKYGAHSGTCPASNHVAGAAALILSKHPNWTNTQVRSSLENTATKLGDSFYYGKGLINVEAAAQHHHHHH

SEQ ID NO: 6 - protein, 31 aa, Artificial Sequence
  liraglutide
  MOD_RES (20)..(20): Lys is Lys(Pal-gamma-Glu)
HAEGTFTSDVSSYLEGQAAKEFIAWLVRGRG

SEQ ID NO: 7 - protein, 31 aa, Artificial Sequence
  semaglutide
  MOD_RES (2)..(2): Aib
  MOD_RES (20)..(20): Lys is Lys(AEEA-AEEA-gamma-Glu-17-carboxyheptadecanoyl)
HXEGTFTSDVSSYLEGQAAKEFIAWLVRGRG

SEQ ID NO: 8 - protein, 29 aa, Artificial Sequence
  dasiglucagon
  MOD_RES (16)..(16): Aib
HSQGTFTSDYSKYLDXARAEEFVKWLEST

SEQ ID NO: 9 - protein, 39 aa, Artificial Sequence
  glepaglutide
  MOD_RES (39)..(39): AMIDATION C-terminal
HGEGTFSSELATILDALAARDFIAWLIATKITDKKKKKK

SEQ ID NO: 10 - protein, 39 aa, Artificial Sequence
  elsiglutide
  MOD_RES (39)..(39): AMIDATION C-terminal
HGEGSFSSELSTILDALAARDFIAWLIATKITDKKKKKK

SEQ ID NO: 11 - protein, 34 aa, Artificial Sequence
  teriparatide
  MOD_RES (1)..(1): N-terminal phenylacetylation might be present in the teriparatide precursor
SVSEIQLMHNLGKHLNSMERVEWLRKKLQDVHNF

SEQ ID NO: 12 - protein, 32 aa, Salmo salar
  DISULFID (1)..(7)
  MOD_RES (32)..(32): AMIDATION C-terminal
CSNLSTCVLGKLSQELHKLQTYPRTNTGSGTP

SEQ ID NO: 13 - protein, 20 aa, artificial sequence
  bivalirudin
  MOD_RES (1)..(1): D-Phe
XPRPGGGGNGDFEEIPEEYL

SEQ ID NO: 14 - protein, 8 aa, Artificial sequence
  8-mer model peptide
  MOD_RES (1)..(1): ACETYLATION N-terminal
  MOD_RES (8)..(8): AMIDATION C-terminal
DFSKLALR

SEQ ID NO: 15 - protein, 8 aa, Artificial Sequence
  Dasi 1-8
  MOD_RES (8)..(8): C-terminal (thio)ester
HSQGTFTS

SEQ ID NO: 16 - protein, 21 aa, Artificial Sequence
  Dasi 9-29
  MOD_RES (8)..(8): Aib
DYSKYLDXARAEEFVKWLEST

SEQ ID NO: 17 - protein, 9 aa, Artificial Sequence
  Dasi 1-9
  MOD_RES (9)..(9): C-terminal (thio)ester
HSQGTFTSD

SEQ ID NO: 18 - protein, 20 aa, Artificial Sequence
  Dasi 10-29
  MOD_RES (7)..(7): Aib
YSKYLDXARAEEFVKWLEST

SEQ ID NO: 19 - protein, 10 aa, Artificial Sequence
  Dasi 1-10
  MOD_RES (10)..(10): C-terminal (thio)ester
HSQGTFTSDY

SEQ ID NO: 20 - protein, 19 aa, Artificial Sequence
  Dasi 11-29
  MOD_RES (6)..(6): Aib
SKYLDXARAEEFVKWLEST

SEQ ID NO: 21 - protein, 11 aa, Artificial Sequence
  Glepa 1-11
  MOD_RES (11)..(11): C-terminal (thio)ester
HGEGTFSSELA

SEQ ID NO: 22 - protein, 28 aa, Artificial Sequence
  Glepa 12-39
TILDALAARDFIAWLIATKITDKKKKKK

SEQ ID NO: 23 - protein, 16 aa, Artificial Sequence
  Glepa 1-16
  MOD_RES (16)..(16): C-terminal (thio)ester
HGEGTFSSELATILDA

SEQ ID NO: 24 - protein, 23 aa, Artificial Sequence
  Glepa 17-39
LAARDFIAWLIATKITDKKKKKK

SEQ ID NO: 25 - protein, 11 aa, Artificial Sequence
  Elsi 1-11
  MOD_RES (11)..(11): C-terminal (thio)ester
HGEGSFSSELS

SEQ ID NO: 26 - protein, 28 aa, Artificial Sequence
  Elsi 12-39
TILDALAARDFIAWLIATKITDKKKKKK

SEQ ID NO: 27 - protein, 16 aa, Artificial Sequence
  Elsi 1-16
  MOD_RES (16)..(16): C-terminal (thio)ester
HGEGSFSSELSTILDA

SEQ ID NO: 28 - protein, 23 aa, Artificial Sequence
  Elsi 17-39
LAARDFIAWLIATKITDKKKKKK

SEQ ID NO: 29 - protein, 11 aa, Artificial Sequence
  Teri 1-11
  MOD_RES (11)..(11): C-terminal (thio)ester
SVSEIQLMHNL

SEQ ID NO: 30 - protein, 23 aa, Artificial Sequence
  Teri 12-34
GKHLNSMERVEWLRKKLQDVHNF

SEQ ID NO: 31 - protein, 12 aa, Artificial Sequence
  Calci 1-12
  MOD_RES (12)..(12): C-terminal (thio)ester
CSNLSTCVLGKL

SEQ ID NO: 32 - protein, 20 aa, Artificial Sequence
  Calci 13-32
  MOD_RES (20)..(20): AMIDATION C-terminal might be present
SQELHKLQTYPRTNTGSGTP

SEQ ID NO: 33 - protein, 20 aa, Artificial Sequence
  Calci 1-20
  MOD_RES (20)..(20): C-terminal (thio)ester
CSNLSTCVLGKLSQELHKLQ

SEQ ID NO: 34 - protein, 12 aa, Artificial Sequence
  Calci 21-32
TYPRTNTGSGTP

SEQ ID NO: 35 - protein, 10 aa, Artificial Sequence
  Biva 1-10
  MOD_RES (1)..(1): D-Phe
  MOD_RES (10)..(10): C-terminal (thio)ester
XPRPGGGGNG

SEQ ID NO: 36 - protein, 10 aa, Artificial Sequence
  Biva 11-20
DFEEIPEEYL

SEQ ID NO: 37 - protein, 11 aa, Artificial Sequence
  Lira-Sema 1-11
  VARIANT (2)..(2): Ala or Aib
  MOD_RES (11)..(11): C-terminal (thio)ester
HXEGTFTSDVS

SEQ ID NO: 38 - protein, 20 aa, Artificial Sequence
  Lira-Sema 12-31
  MOD_RES (9)..(9): Lys is selected from Lys, Lys(PG), Lys(gamma-Glu), Lys(Pal-gamma-Glu) and Lys(AEEA-AEEA-gamma-Glu-17-carboxyheptadecanoyl)
SYLEGQAAKEFIAWLVRGRG

SEQ ID NO: 39 - protein, 11 aa, Artificial Sequence
  Lira 1-11
  MOD_RES (11)..(11): C-terminal  -OCam-Phe-Lys-NH2 ester
HAEGTFTSDVS

SEQ ID NO: 40 - protein, 20 aa, Artificial Sequence
  Lira 12-31
  MOD_RES (9)..(9): Lys is Lys(Pal-gamma-Glu)
SYLEGQAAKEFIAWLVRGRG

SEQ ID NO: 41 - protein, 5 aa, Artificial Sequence
  model peptide fragment
  MOD_RES (1)..(1): ACETYLATION N-terminal
  MOD_RES (5)..(5): C-terminal  -OCam-Leu-OH ester or OH
DFSKL

SEQ ID NO: 42 - protein, 42 aa, Artificial Sequence
  lira 1-11-1-31
  MOD_RES (31)..(31): Lys is Lys(Pal-gamma-Glu)
HAEGTFTSDVSHAEGTFTSDVSSYLEGQAAKEFIAWLVRGRG

SEQ ID NO: 43 - protein, 11 aa, Artificial Sequence
  Teri 1-11 ester
  MOD_RES (1)..(1): N-terminal phenylacetilation
  MOD_RES (11)..(11): C-terminal -OCam-Leu-OH ester
SVSEIQLMHNL

SEQ ID NO: 44 - protein, 11 aa, Artificial Sequence
  Sema 1-11
  MOD_RES (2)..(2): Aib
  MOD_RES (11)..(11): C-terminal -OCam-Phe-Lys-NH2 ester
HXEGTFTSDVS

SEQ ID NO: 45 - protein, 20 aa, Artificial Sequence
  Sema 12-31
  MOD_RES (9)..(9): Lys is Lys(AEEA-AEEA-gamma-Glu-17-carboxyheptadecanoyl)
SYLEGQAAKEFIAWLVRGRG